European Patent Specification EP 4 161 954 B1, published November 1, 2023. Title: SERUM STABLE BINDING PROTEINS FOR HUMAN HER2 FOR THERANOSTIC APPLICATIONS. Applicant: Navigo Proteins GmbH. The sequence listing filed with the application follows.

SEQUENCE LISTING (18 sequences)

SEQ ID NO: 1 - protein, 152 aa, Artificial Sequence
  206478
MQIFVKTLTGKTITLEVEPSDTTENVKAKIQDKEGIPPDQQTLAFVGKQLEDGRTLSDYNIQKESTLWLYLTLRAAMRIFVKTHTGKTITLDVEPSDTIENVKAKIQDKEGIPPDQQRLIWAGKQLEDGRTLSDYNIQEWSILHLVLRLRAA

SEQ ID NO: 2 - protein, 152 aa, Artificial Sequence
  206479
MQIFVKTLTGKTITLEVEPSDTTENVKAKIQDKEGIPPDQQTLAFVGKQLEDGRTLSDYNIQKESTLWLYLTLRAAMRIFVKTHTGKTITLDVEPSDTIENVKAKIQDKEGIPPDQQRLIWAGKQLEDGRTLSDYNIQEWAILHLVLRLRAA

SEQ ID NO: 3 - protein, 152 aa, Artificial Sequence
  206480
MQIFVKTLTGKTITLEVEPSDTTENVKAKIQDKEGIPPDQQTLAFVGKQLEDGRTLSDYNIQKESTLWLYLTLRAAMRIFVKTHTGKTITLDVEPSDTIENVKAKIQDKEGIPPDQQRLIWAGKQLEDGRTLSDYNISEWSILHLVLRLRAA

SEQ ID NO: 4 - protein, 152 aa, Artificial Sequence
  206494
MQIFVKTLTGKTITLEVEPSDTTENVKAKIQDKEGIPPDQQTLAFVGKQLEDGRTLSDYNIQKESTLWLYLTWRAAMRIFVKTHTGKTITLDVEPSDTIENVKAKIQDKEGIPPDQQRLIWAGKQLEDGRTLSDYNIQEWSILHLVLRLRAA

SEQ ID NO: 5 - protein, 152 aa, Artificial Sequence
  206486
MQIFVKTLTGKTITLEVEPSDTTENVKAKIQDKEGIPPDQQTLAFVGKQLEDGRTLSDYNIQKESTLWLYLTLYAAMRIFVKTHTGKTITLDVEPSDTIENVKAKIQDKEGIPPDQQRLIWAGKQLEDGRTLSDYNIQEWSILHLVLRLRAA

SEQ ID NO: 6 - protein, 152 aa, Artificial Sequence
  206482
MQIFVKTLTGKTITLEVEPSDTTENVKAKIQDKEGIPPDQQTLAFVGKQLEDGRTLSDYNIQKESTLWLYLTLRAAMRIFVTTHTGKTITLDVEPSDTIENVKAKIQDKEGIPPDQQRLIWAGKQLEDGRTLSDYNIQEWSILHLVLRLRAA

SEQ ID NO: 7 - protein, 152 aa, Artificial Sequence
  206483
MQIFVKTLTGKTITLEVEPSDTTENVKAKIQDKEGIPPDQQTLAFVGKQLEDGRTLSDYNIQKESTLWLYLTLRAAMRIFVTTHTGKTITLDVEPSDTIENVKAKIQDKEGIPPDQQRLIWAGKQLEDGRTLSDYNIQEWAILHLVLRLRAA

SEQ ID NO: 8 - protein, 152 aa, Artificial Sequence
  206498
MQIFVKTLTGKTITLEVEPSDTTENVKAKIQDKEGIPPDQQTLAFVGKQLEDGRTLSDYNIQKESTLWLYLTWRAAMRIFVTTHTGKTITLDVEPSDTIENVKAKIQDKEGIPPDQQRLIWAGKQLEDGRTLSDYNIQEWSILHLVLRLRAA

SEQ ID NO: 9 - protein, 152 aa, Artificial Sequence
  206481
MQIFVKTLTGKTITLEVEPSDTTENVKAKIQDKEGIPPDQQTLAFVGKQLEDGRTLSDYNIQKESTLWLYLTLRAAMRIFVKTHTGKTITLDVEPSDTIENVKAKIQDKEGIPPDQQRLIWAGKQLEDGRTLSDYNISEWAILHLVLRLRAA

SEQ ID NO: 10 - protein, 152 aa, Artificial Sequence
  206495
MQIFVKTLTGKTITLEVEPSDTTENVKAKIQDKEGIPPDQQTLAFVGKQLEDGRTLSDYNIQKESTLWLYLTWRAAMRIFVKTHTGKTITLDVEPSDTIENVKAKIQDKEGIPPDQQRLIWAGKQLEDGRTLSDYNIQEWAILHLVLRLRAA

SEQ ID NO: 11 - protein, 152 aa, Artificial Sequence
  206504
MQIFVKTLTGKTITLEVEPSDTTENVKAKIQDKEGIPPDQQTLAFVGKQLEDGRTLSDYNIQKESTLWLYLTWYAAMRIFVKTHTGKTITLDVEPSDTIENVKAKIQDKEGIPPDQQRLIWAGKQLEDGRTLSDYNISEWSILHLVLRLRAA

SEQ ID NO: 12 - protein, 152 aa, Artificial Sequence
  206485
MQIFVKTLTGKTITLEVEPSDTTENVKAKIQDKEGIPPDQQTLAFVGKQLEDGRTLSDYNIQKESTLWLYLTLRAAMRIFVTTHTGKTITLDVEPSDTIENVKAKIQDKEGIPPDQQRLIWAGKQLEDGRTLSDYNISEWAILHLVLRLRAA

SEQ ID NO: 13 - protein, 152 aa, Artificial Sequence
  206499
MQIFVKTLTGKTITLEVEPSDTTENVKAKIQDKEGIPPDQQTLAFVGKQLEDGRTLSDYNIQKESTLWLYLTWRAAMRIFVTTHTGKTITLDVEPSDTIENVKAKIQDKEGIPPDQQRLIWAGKQLEDGRTLSDYNIQEWAILHLVLRLRAA

SEQ ID NO: 14 - protein, 152 aa, Artificial Sequence
  206497
MQIFVKTLTGKTITLEVEPSDTTENVKAKIQDKEGIPPDQQTLAFVGKQLEDGRTLSDYNIQKESTLWLYLTWRAAMRIFVKTHTGKTITLDVEPSDTIENVKAKIQDKEGIPPDQQRLIWAGKQLEDGRTLSDYNISEWAILHLVLRLRAA

SEQ ID NO: 15 - protein, 152 aa, Artificial Sequence
  her2 binding protein
  Xaa (73)..(73): Xaa may be selected from L or W
  Xaa (74)..(74): Xaa may be selected from R or Y
  Xaa (82)..(82): Xaa may be selected from K or T
  Xaa (138)..(138): Xaa may be selected from Q or S
  Xaa (141)..(141): Xaa may be selected from S or A
MQIFVKTLTGKTITLEVEPSDTTENVKAKIQDKEGIPPDQQTLAFVGKQLEDGRTLSDYNIQKESTLWLYLTXXAAMRIFVXTHTGKTITLDVEPSDTIENVKAKIQDKEGIPPDQQRLIWAGKQLEDGRTLSDYNIXEWXILHLVLRLRAA

SEQ ID NO: 16 - protein, 152 aa, Artificial Sequence
  wt ubiquitin dimer
MQIFVKTLTGKTITLEVEPSDTIENVKAKIQDKEGIPPDQQRLIFAGKQLEDGRTLSDYNIQKESTLHLVLRLRAAMQIFVKTLTGKTITLEVEPSDTIENVKAKIQDKEGIPPDQQRLIFAGKQLEDGRTLSDYNIQKESTLHLVLRLRAA

SEQ ID NO: 17 - protein, 58 aa, Artificial Sequence
  PAdelFc
IAAQHDKIQQAADKEILHLPNLTEEQRNKFRQSLRDDPSVSAEILAEAKKLNDAQAPK

SEQ ID NO: 18 - protein, 412 aa, Artificial Sequence
  fusion protein of SEQ2 with IgG  (209438) n[UbFrag_(G4S)x4_mIgG2a-Fc_SA-Strep]c
MQIFVKTLTGKTITLEVEPSDTTENVKAKIQDKEGIPPDQQTLAFVGKQLEDGRTLSDYNIQKESTLWLYLTLRAAMRIFVKTHTGKTITLDVEPSDTIENVKAKIQDKEGIPPDQQRLIWAGKQLEDGRTLSDYNIQEWAILHLVLRLRAAGGGGSGGGGSGGGGSGGGGSGPTIKPCPPCKCPAPNLLGGPSVFIFPPKIKDVLMISLSPIVTCVVVDVSEDDPDVQISWFVNNVEVHTAQTQTHREDYNSTLRVVSALPIQHQDWMSGKEFKCKVNNKDLPAPIERTISKPKGSVRAPQVYVLPPPEEEMTKKQVTLTCMVTDFMPEDIYVEWTNNGKTELNYKNTEPVLDSDGSYFMYSKLRVEKKNWVERNSYSCSVVHEGLHNHHTTKSFSCTPGKSAWSHPQFEK